European Patent Application EP 4 582 089 A2, published July 9, 2025. Title: PARTICLE-MEDIATED DELIVERY OF BIOLOGICS. Applicant: MAYO FOUNDATION FOR MEDICAL EDUCATION AND RESEARCH. Application EP, filed November 22, 2017. The sequence listing filed with the application follows.

SEQUENCE LISTING (14 sequences)

SEQ ID NO: 1 - DNA, 70 bp, synthetic construct
  misc_feature 1..70: note = Internal ribosome entry site
  source 1..70: mol_type = other DNA
cccattgtatgggatctgatctggggcctcggtgcacatgctttacatgtgtttagtcgaggttaaaaaa

SEQ ID NO: 2 - DNA, 47 bp, synthetic construct
  misc_feature 1..47: note = Internal ribosome entry site
  source 1..47: mol_type = other DNA
acgtctaggccccccgaaccacggggacgtggttttcctttgaaaaa

SEQ ID NO: 3 - DNA, 138 bp, synthetic construct
  misc_feature 1..138: note = Internal ribosome entry site
  source 1..138: mol_type = other DNA
ccagaaggtaccccattgtatgggatctgatctggggcctcggtacacatgctttacatgtgtttagtcgaggttaaaaaaacgtctaggccccccgaaccacggggacgtggttttcctttgaaaaacacgatgata

SEQ ID NO: 4 - DNA, 173 bp, synthetic construct
  misc_feature 1..173: note = Internal ribosome entry site
  source 1..173: mol_type = other DNA
atatggccacaaccatggtgagcaagggcgaggagctgttcaccggggtggtgcccatcctggtcgagctggacggcgacgtaaacggccacaagttcagcgtgtccggcgagggcgagggcgatgccacctacggcaagctgaccctgaagttcatctgcaccaccggcaag

SEQ ID NO: 5 - DNA, 265 bp, synthetic construct
  misc_feature 1..265: note = Internal ribosome entry site
  misc_feature 26: note = n is a, c, g, or t
  misc_feature 30: note = n is a, c, g, or t
  misc_feature 167..169: note = n is a, c, g, or t
  misc_feature 187..188: note = n is a, c, g, or t
  misc_feature 197..199: note = n is a, c, g, or t
  misc_feature 204..215: note = n is a, c, g, or t
  source 1..265: mol_type = other DNA
gctgctgcccgacaaccactacctgnagcnacccagtccgccctgagcaaagaccccaacgagaagcgcgatcacatggtcctgctggagttcgtgaccgccgccgggatcactctcggcatggacgagctgtacaagtaagccctgtggaatgtgtgtcagttagnnnggtgtggaaagtccccannggctccccnnnagcannnnnnnnnnnnggcagaagtatgcaaagcatgcatctcaattagtcagcaaccaggtgtgg

SEQ ID NO: 6 - DNA, 160 bp, synthetic construct
  misc_feature 1..160: note = Internal ribosome entry site
  misc_feature 41..43: note = n is a, c, g, or t
  misc_feature 125: note = n is a, c, g, or t
  misc_feature 148..149: note = n is a, c, g, or t
  source 1..160: mol_type = other DNA
caacgtctatatcatggccgacaagcagaagaacggcatcnnnaaggtgaacttcaagatccgccacaacatcgaggacggcagcgtgcagctcgccgaccactaccagcagaacacccccatcnggcgacggccccgtgctgctgcnnccgacaaccac

SEQ ID NO: 7 - DNA, 160 bp, synthetic construct; identical to SEQ ID NO: 6
  misc_feature 1..160: note = Internal ribosome entry site
  misc_feature 41..43: note = n is a, c, g, or t
  misc_feature 125: note = n is a, c, g, or t
  misc_feature 148..149: note = n is a, c, g, or t
  source 1..160: mol_type = other DNA

SEQ ID NO: 8 - DNA, 136 bp, synthetic construct
  misc_feature 1..136: note = Internal ribosome entry site
  misc_feature 28..29: note = n is a, c, g, or t
  misc_feature 56: note = n is a, c, g, or t
  misc_feature 95..97: note = n is a, c, g, or t
  misc_feature 119..121: note = n is a, c, g, or t
  source 1..136: mol_type = other DNA
gctgaagcactgcacgccgtaggtcagnnggtggtcacgagggtgggccagggcancgggcagcttgccggtggtgcagatgaacttcagggtcnnnagcttgccgtaggtggcatcgnnnccctcgccctcgccg

SEQ ID NO: 9 - DNA, 235 bp, synthetic construct
  misc_feature 1..235: note = Internal ribosome entry site
  misc_feature 55..57: note = n is a, c, g, or t
  misc_feature 94..96: note = n is a, c, g, or t
  misc_feature 194: note = n is a, c, g, or t
  source 1..235: mol_type = other DNA
gacacgctgaacttgtggccgtttacgtcgccgtccagctcgaccaggatgggcnnnaccaccccggtgaacagctcctcgcccttgctcaccnnnatggttgtggccatattatcatcgtgtttttcaaaggaaaaccacgtccccgtggttcggggggcctagacgtttttttaacctcgactaaacacatngtaaagcatgtgtaccgaggccccagatcagatcccataca

SEQ ID NO: 10 - DNA, 389 bp, synthetic construct
  misc_feature 1..389: note = Internal ribosome entry site
  misc_feature 80..82: note = n is a, c, g, or t
  misc_feature 101..106: note = n is a, c, g, or t
  misc_feature 126..133: note = n is a, c, g, or t
  misc_feature 138..146: note = n is a, c, g, or t
  misc_feature 175..176: note = n is a, c, g, or t
  misc_feature 201: note = n is a, c, g, or t
  misc_feature 205..209: note = n is a, c, g, or t
  misc_feature 234..243: note = n is a, c, g, or t
  misc_feature 252..255: note = n is a, c, g, or t
  misc_feature 264: note = n is a, c, g, or t
  misc_feature 270: note = n is a, c, g, or t
  misc_feature 313..316: note = n is a, c, g, or t
  misc_feature 343..353: note = n is a, c, g, or t
  source 1..389: mol_type = other DNA
agggcacgggcagcttgccggtggtgcagatgaacttcagggtcagcttgccgtaggtggcatcgccctcgccctcgccnnnggacacgctgaacttgtgnnnnnngccgtttacgtcgccgtccnnnnnnnnagctnnnnnnnnncgaccaggatgggcaccaccccggtgaanncagctcctcgcccttgctcaccatnggtnnnnntgtggccatattatcatcgtgtttnnnnnnnnnnttcaaaggnnnnaaaaccacngtcccncgtggttcggggggcctagacgtttttttaacctcgactaaannnncacatgtaaagcatgtgtaccgaggcnnnnnnnnnnncccagatcagatcccatacaatggggtaccttctgg

SEQ ID NO: 11 - RNA, 19 nt, Synthetic construct
  source 1..19: mol_type = transcribed RNA
aaaaaaaaaaaaaaaaaaa

SEQ ID NO: 12 - RNA, 13 nt, Synthetic construct
  source 1..13: mol_type = transcribed RNA
ttttttttttttt

SEQ ID NO: 13 - RNA, 28 nt, Synthetic construct
  source 1..28: mol_type = transcribed RNA
aaaaaaaaaaaaaaaaaaaaaaaaaaaa

SEQ ID NO: 14 - RNA, 16 nt, Synthetic construct
  source 1..16: mol_type = transcribed RNA
tttttttttttttttt